European Patent Application EP 4 545 550 A1, published April 30, 2025. Title: INSECT NEUROPEPTIDES 3. Applicant: SOLASTA Bio Limited. The sequence listing filed with the application follows.

SEQUENCE LISTING (16 sequences)

SEQ ID NO: 1 - protein, 16 aa, synthetic construct
  source 1..16: note = Z peptide
NADEDQQQSVDFTPRL

SEQ ID NO: 2 - protein, 16 aa, synthetic construct
  source 1..16: note = SB-P-80
  MOD_RES 16: note = leucinamide
NADEDQQQSVDFTPRL

SEQ ID NO: 3 - protein, 11 aa, synthetic construct
  source 1..11: note = SB-P-47
  MOD_RES 11: note = leucinamide
  MOD_RES 1: note = pyroglutamyl-alanine
AIMARPQVPRL

SEQ ID NO: 4 - protein, 8 aa, synthetic construct
  source 1..8: note = SB-P-49
  MOD_RES 8: note = leucinamide
SVPFKPRL

SEQ ID NO: 5 - protein, 19 aa, synthetic construct
  source 1..19: note = SB-P-51
  MOD_RES 19: note = leucinamide
LRQLQSNGEPAYRVRTPRL

SEQ ID NO: 6 - protein, 12 aa, synthetic construct
  source 1..12: note = SB-P-46
  MOD_RES 12: note = leucinamide
SPPYSPPFSPRL

SEQ ID NO: 7 - protein, 10 aa, synthetic construct
  source 1..10: note = SB-P-81
  MOD_RES 10: note = leucinamide
GGSMTFSPRL

SEQ ID NO: 8 - protein, 8 aa, synthetic construct
  source 1..8: note = SB-P-70
  MOD_RES 8: note = glycinamide
KVKFSAWG

SEQ ID NO: 9 - protein, 10 aa, synthetic construct
  source 1..10: note = SB-P-65
  MOD_RES 10: note = glycinamide
RQKTVFSSWG

SEQ ID NO: 10 - protein, 7 aa, synthetic construct
  source 1..7: note = SB-P-66
  MOD_RES 7: note = glycinamide
PAFSSWG

SEQ ID NO: 11 - protein, 9 aa, synthetic construct
  source 1..9: note = SB-P-86
  MOD_RES 9: note = glycinamide
  MOD_RES 1: note = pyroglutamyl-leucine
LTFTSSWGG

SEQ ID NO: 12 - protein, 8 aa, synthetic construct
  source 1..8: note = SB-P-039
  MOD_RES 1: note = palmitoyl-glutamine
  MOD_RES 8: note = tryptophanamide
QLTFSPDW

SEQ ID NO: 13 - protein, 7 aa, synthetic construct
  source 1..7: note = SB-P-042
  MOD_RES 1: note = pyroglutamyl-leucine
  MOD_RES 7: note = tryptophanamide
LTFSPDW

SEQ ID NO: 14 - protein, 6 aa, synthetic construct
  source 1..6: note = SB-P-69
  MOD_RES 6: note = glycinamide
NFSPWG

SEQ ID NO: 15 - protein, 19 aa, synthetic construct
  source 1..19: note = SB-P-48
  MOD_RES 19: note = leucinamide
EQNVQSNGEPAYRVRTPRL

SEQ ID NO: 16 - protein, 8 aa, synthetic construct
  source 1..8: note = SB-P-41
  MOD_RES 8: note = tryptophanamide
QLTFSPDW